European Patent Application EP 4 190 814 A1, published June 7, 2023. Title: METHODS OF USING BISPECIFIC CD33 AND CD3 BINDING PROTEINS. Applicant: Amphivena Therapeutics, Inc. Application EP. The sequence listing filed with the application follows.

SEQUENCE LISTING (146 sequences)

SEQ ID NO: 1 - protein, 108 aa, Homo sapiens
SYELTQPPSVSVAPGQTAMITCGGNNIGSTTVHWYQQKPGQAPVLVVYDDNERPSGIPERFSGSNSGSTATLTINRVEAGDEADYYCQVWDSGSDHVVFGGGTKLTVL

SEQ ID NO: 2 - protein, 110 aa, Homo sapiens
QSVLTQPPSASGTPGQRVTISCSGSRSNIGSNTVNWYQQLPGTAPKLLIYGNNQRPSGVPDRFSGSKSGSSASLAISGLQSEDEADYYCATWDDSLIGWVFGGGTKLTVL

SEQ ID NO: 3 - protein, 110 aa, Homo sapiens
QSVLTQPPSASGTPGQRVTISCSGSRSNIGSNTVNWYQQLPGTAPKLLIYGNNQRPSGVPDRFSGSKSGTSASLAISGLQSEDEADYYCATWDDSLIGWVFGGGTKLTVL

SEQ ID NO: 4 - protein, 110 aa, Homo sapiens; identical to SEQ ID NO: 3

SEQ ID NO: 5 - protein, 110 aa, Homo sapiens; identical to SEQ ID NO: 3

SEQ ID NO: 6 - protein, 110 aa, Homo sapiens
QSVLTQPPSASGTPGQRVTISCSGSSSNIGSNTVNWYQQLPGTAPKLLIYSDNQRPSGVPDRFSGSKSGSSASLAISGLQSDDEADYYCATWDDSLNGAVFGGGTKLTVL

SEQ ID NO: 7 - protein, 111 aa, Homo sapiens
QSVLTQPPSVSGAPGQRVTISCTGSSSNIGAGYDVHWYQQLPGTAPKLLIYGNSNRPSGVPDRFSGSKSGTSASLAITGLQAEDEADYYCQSYDSSLSDVVFGGGTKLTVL

SEQ ID NO: 8 - protein, 110 aa, Homo sapiens
QSVLTQPPSASGTPGQRVTISCSGSSSNIGSNIVNWYQQLPGTAPKLLIYSNNQRPSGVPDRFSGSKSGTSASLAISGLQSEDEADYYCAAWDDSLKGYVFGGGTKLTVL

SEQ ID NO: 9 - protein, 110 aa, Homo sapiens
QSVLTQPPSASGTPGQRVTISCSGSSSNIGSNTVKWYQQLPGTAPKLLIYSNNQRSSGVPDRFSGSKSGSSASLAISGLQSEDEADYYCAAWDDSLNGYVFGGGTKLTVL

SEQ ID NO: 10 - protein, 110 aa, Homo sapiens
QSVLTQPPSASGTPGQRVTISCSGSSSNIGDNVVNWYQQLPGTAPKLLIYSTNKRPSGVPDRFSGSKSGSSASLAISGLQSEDEADYYCAAWDDSLSAYVFGGGTKLTVL

SEQ ID NO: 11 - protein, 119 aa, Homo sapiens
QVQLQESGGGVVQPGRSLRLSCAASGFSFSNYGIHWVRQAPGKGLEWVALISYDGNKKFYADSVKGRFAISRDTSKNTVDLQMTSLRPEDTAVYYCAKDRLESAAFDYWGQGTLVTVSS

SEQ ID NO: 12 - protein, 122 aa, Homo sapiens
QVQLVQSGAEVKKPGASVKVSCKASGYTFTSYDINWVRQAPGQGLEWMGWMNPNSGNTGFAQKFQGRVTMTRDTSTSTVYMELSSLRSEDTAVYYCARDRANTDFSYGMDVWGQGTLVTVSS

SEQ ID NO: 13 - protein, 122 aa, Homo sapiens
QVQLVQSGAEVKKPGASVKVSCKASGYTFTSYDINWVRQAPGQGLEWMGWMNPNSGNTGFAQKFQGRVTMTRDTSTSTVYMELSSLRSEDTAVYYCARDRAVTDYYYGMDVWGQGTLVTVSS

SEQ ID NO: 14 - protein, 122 aa, Homo sapiens
QVQLVQSGAEVKKPGASVKVSCKASGYTFTSYDINWVRQAPGQGLEWMGWMNPNSGNTGFAQKFQGRVTMTRDTSTSTVYMELSSLRSEDTAVYYCARDRANTDYSFGMDVWGQGTLVTVSS

SEQ ID NO: 15 - protein, 122 aa, Homo sapiens
QVQLVQSGAEVKKPGASVKVSCKASGYTFTSYDINWVRQAPGQGLEWMGWMNPNSGNTGFAQKFQGRVTMTRDTSTSTVYMELSSLRSEDTAVYYCARDRANTDYSLGMDVWGQGTLVTVSS

SEQ ID NO: 16 - protein, 123 aa, Homo sapiens
QVQLVQSGAEVKKPGASVKVSCKASGYTFTSYYMHWVRQAPGQGLEWMGIINPSGGSTSYAQKFQGRVTMTRDTSTSTVYMELSSLRSEDTAVYYCARDVVPAAIDYYGMDVWGQGTTVTVSS

SEQ ID NO: 17 - protein, 119 aa, Homo sapiens
QVQLVQSGAEVKKPGESLKISCKGSGYSFTSYWIGWVRQMPGKGLEWMGIIYPGDSDTRYSPSFQGQVTISADKSISTAYLQWSSLKASDTAMYYCARHKRGSDAFDIWGQGTTVTVSS

SEQ ID NO: 18 - protein, 122 aa, Homo sapiens
QVQLVQSGAEVKKPGSSVKVSCKASGGTFSSYAISWVRQAPGQGLEWMGGIYPIFGSANYAQKFQGRVTITADESTSTAYMELSSLRSEDTAVYYCAREYYYDSSEWAFDIWGQGTLVTVSS

SEQ ID NO: 19 - protein, 122 aa, Homo sapiens
QVQLVQSGAEVKKPGSSVKVSCKASGGTFSSYGISWVRQAPGQGLEWMGGIIPIFGSAHYAQKFQGRVTITADESTSTAYMELSSLRSEDTAVYYCAREYYYDSSEWAFDIWGQGTLVTVSS

SEQ ID NO: 20 - protein, 122 aa, Homo sapiens
QVQLVQSGAEVKKPGSSVKVSCKASGGTFDSYAISWVRQAPGQGLEWMGGIIPIFGSAHYSQKFQGRVTITADESTSTAYMELSSLRSEDTAVYYCAREYYYDSSEWAFDIWGQGTLVTVSS

SEQ ID NO: 21 - protein, 11 aa, Homo sapiens
GGNNIGSTTVH

SEQ ID NO: 22 - protein, 13 aa, Homo sapiens
SGSRSNIGSNTVN

SEQ ID NO: 23 - protein, 13 aa, Homo sapiens
SGSSSNIGSNTVN

SEQ ID NO: 24 - protein, 14 aa, Homo sapiens
TGSSSNIGAGYDVH

SEQ ID NO: 25 - protein, 13 aa, Homo sapiens
SGSSSNIGSNIVN

SEQ ID NO: 26 - protein, 13 aa, Homo sapiens
SGSSSNIGSNTVK

SEQ ID NO: 27 - protein, 13 aa, Homo sapiens
SGSSSNIGDNVVN

SEQ ID NO: 28 - protein, 7 aa, Homo sapiens
DDNERPS

SEQ ID NO: 29 - protein, 7 aa, Homo sapiens
GNNQRPS

SEQ ID NO: 30 - protein, 7 aa, Homo sapiens
SDNQRPS

SEQ ID NO: 31 - protein, 7 aa, Homo sapiens
GNSNRPS

SEQ ID NO: 32 - protein, 7 aa, Homo sapiens
SNNQRPS

SEQ ID NO: 33 - protein, 7 aa, Homo sapiens
SNNQRSS

SEQ ID NO: 34 - protein, 7 aa, Homo sapiens
STNKRPS

SEQ ID NO: 35 - protein, 9 aa, Homo sapiens
QVWDSGSDH

SEQ ID NO: 36 - protein, 9 aa, Homo sapiens
ATWDDSLIG

SEQ ID NO: 37 - protein, 9 aa, Homo sapiens
ATWDDSLNG

SEQ ID NO: 38 - protein, 9 aa, Homo sapiens
QSYDSSLSD

SEQ ID NO: 39 - protein, 9 aa, Homo sapiens
AAWDDSLKG

SEQ ID NO: 40 - protein, 9 aa, Homo sapiens
AAWDDSLNG

SEQ ID NO: 41 - protein, 9 aa, Homo sapiens
AAWDDSLSA

SEQ ID NO: 42 - protein, 6 aa, Homo sapiens
SNYGIH

SEQ ID NO: 43 - protein, 6 aa, Homo sapiens
TSYDIN

SEQ ID NO: 44 - protein, 6 aa, Homo sapiens
TSYYMH

SEQ ID NO: 45 - protein, 6 aa, Homo sapiens
TSYWIG

SEQ ID NO: 46 - protein, 6 aa, Homo sapiens
SSYAIS

SEQ ID NO: 47 - protein, 6 aa, Homo sapiens
SSYGIS

SEQ ID NO: 48 - protein, 6 aa, Homo sapiens
DSYAIS

SEQ ID NO: 49 - protein, 17 aa, Homo sapiens
LISYDGNKKFYADSVKG

SEQ ID NO: 50 - protein, 17 aa, Homo sapiens
WMNPNSGNTGFAQKFQG

SEQ ID NO: 51 - protein, 18 aa, Homo sapiens
GIINPSGGSTSYAQKFQG

SEQ ID NO: 52 - protein, 17 aa, Homo sapiens
IIYPGDSDTRYSPSFQG

SEQ ID NO: 53 - protein, 17 aa, Homo sapiens
GIYPIFGSANYAQKFQG

SEQ ID NO: 54 - protein, 17 aa, Homo sapiens
GIIPIFGSAHYAQKFQG

SEQ ID NO: 55 - protein, 17 aa, Homo sapiens
GIIPIFGSAHYSQKFQG

SEQ ID NO: 56 - protein, 10 aa, Homo sapiens
DRLESAAFDY

SEQ ID NO: 57 - protein, 13 aa, Homo sapiens
DRANTDFSYGMDV

SEQ ID NO: 58 - protein, 13 aa, Homo sapiens
DRAVTDYYYGMDV

SEQ ID NO: 59 - protein, 13 aa, Homo sapiens
DRANTDYSFGMDV

SEQ ID NO: 60 - protein, 13 aa, Homo sapiens
DRANTDYSLGMDV

SEQ ID NO: 61 - protein, 14 aa, Homo sapiens
DVVPAAIDYYGMDV

SEQ ID NO: 62 - protein, 10 aa, Homo sapiens
HKRGSDAFDI

SEQ ID NO: 63 - protein, 13 aa, Homo sapiens
EYYYDSSEWAFDI

SEQ ID NO: 64 - protein, 125 aa, Homo sapiens
EVQLVESGGGLVQPGGSLRLSCAASGFTFSTYAMNWVRQAPGKGLEWVGRIRSKYNNYATYYADSVKDRFTISRDDSKNSLYLQMNSLKTEDTAVYYCARHGNFGNSYVSYFAYWGQGTLVTVSS

SEQ ID NO: 65 - protein, 125 aa, Homo sapiens
EVQLVESGGGLVQPGGSLRLSCAASGFTFSTYAMNWVRQAPGKGLEWVGRIRSKYNNYATYYADSVKDRFTISRDDSKNSLYLQMNSLKTEDTAVYYCARHGNFGNSYVSWFAYWGQGTLVTVSS

SEQ ID NO: 66 - protein, 125 aa, Homo sapiens; identical to SEQ ID NO: 65

SEQ ID NO: 67 - protein, 125 aa, Homo sapiens; identical to SEQ ID NO: 65

SEQ ID NO: 68 - protein, 110 aa, Homo sapiens
DIQMTQSPSSLSASVGDRVTITCRSSTGAVTTSNYANWVQQKPGKAPKALIGGTNKRAPGVPSRFSGSLIGDKATLTISSLQPEDFATYYCALWYSNLWVFGQGTKVEIK

SEQ ID NO: 69 - protein, 110 aa, Homo sapiens
DIQMTQSPSSLSASVGDRVTITCRSSTGAVTTSNYANWVQQKPGKAPKGLIGGTNKRAPGVPARFSGSGSGTDFTLTISSLQPEDFATYYCALWYSNLWVFGQGTKVEIK

SEQ ID NO: 70 - protein, 110 aa, Homo sapiens
DIQMTQSPSSLSASVGDRVTITCRSSTGAVTTSNYANWVQQKPGKAPKGLIGGTNKRAPGVPSRFSGSLIGDKATLTISSLQPEDFATYYCALWYSNLWVFGQGTKVEIK

SEQ ID NO: 71 - protein, 110 aa, Homo sapiens
DIQMTQSPSSLSASVGDRVTITCRSSTGAVTTSNYANWVQQKPGKAPKGLIGGTNKRAPGVPSRFSGSLIGTDFTLTISSLQPEDFATYYCALWYSNLWVFGQGTKVEIK

SEQ ID NO: 72 - protein, 6 aa, Homo sapiens
STYAMN

SEQ ID NO: 73 - protein, 19 aa, Homo sapiens
RIRSKYNNYATYYADSVKD

SEQ ID NO: 74 - protein, 14 aa, Homo sapiens
HGNFGNSYVSWFAY

SEQ ID NO: 75 - protein, 14 aa, Homo sapiens
HGNFGNSYVSYFAY

SEQ ID NO: 76 - protein, 6 aa, Homo sapiens
NTYAMN

SEQ ID NO: 77 - protein, 6 aa, Homo sapiens
NTYAMH

SEQ ID NO: 78 - protein, 6 aa, Homo sapiens
NKYAMN

SEQ ID NO: 79 - protein, 19 aa, Homo sapiens
RIRNKYNNYATYYADSVKD

SEQ ID NO: 80 - protein, 19 aa, Homo sapiens
RIRNKYNNYATEYADSVKD

SEQ ID NO: 81 - protein, 19 aa, Homo sapiens
RIRSKYNNYATEYAASVKD

SEQ ID NO: 82 - protein, 19 aa, Homo sapiens
RIRNKYNNYATEYAASVKD

SEQ ID NO: 83 - protein, 19 aa, Homo sapiens
RIRSKYNNYATYYADSVKG

SEQ ID NO: 84 - protein, 19 aa, Homo sapiens
RIRSKYNNYATEYADSVKS

SEQ ID NO: 85 - protein, 14 aa, Homo sapiens
HGNFGDSYVSWFAY

SEQ ID NO: 86 - protein, 14 aa, Homo sapiens
HGNFGNTYVSWFAY

SEQ ID NO: 87 - protein, 14 aa, Homo sapiens
HGNFGCSYVSWFAY

SEQ ID NO: 88 - protein, 14 aa, Homo sapiens
HGNFGNSYISYWAY

SEQ ID NO: 89 - protein, 14 aa, Homo sapiens
HGNFGNSYVSFFAY

SEQ ID NO: 90 - protein, 14 aa, Homo sapiens
RSSTGAVTTSNYAN

SEQ ID NO: 91 - protein, 7 aa, Homo sapiens
GTNKRAP

SEQ ID NO: 92 - protein, 7 aa, Homo sapiens
ALWYSNL

SEQ ID NO: 93 - protein, 242 aa, Homo sapiens
DPNFWLQVQESVTVQEGLCVLVPCTFFHPIPYYDKNSPVHGYWFREGAIISRDSPVATNKLDQEVQEETQGRFRLLGDPSRNNCSLSIVDARRRDNGSYFFRMERGSTKYSYKSPQLSVHVTDLTHRPKILIPGTLEPGHSKNLTCSVSWACEQGTPPIFSWLSAAPTSLGPRTTHSSVLIITPRPQDHGTNLTCQVKFAGAGVTTERTIQLNVTYVPQNPTTGIFPGDGSGKQETRAGVVH

SEQ ID NO: 94 - protein, 9 aa, Homo sapiens
DQEVQEETQ

SEQ ID NO: 95 - protein, 6 aa, synthetic construct
  REGION 1..6: note = Description of Artificial Sequence: Synthetic peptide
GGSGGS

SEQ ID NO: 96 - protein, 4 aa, synthetic construct
  REGION 1..4: note = Description of Artificial Sequence: Synthetic peptide
GGSG

SEQ ID NO: 97 - protein, 5 aa, synthetic construct
  REGION 1..5: note = Description of Artificial Sequence: Synthetic peptide
GGSGG

SEQ ID NO: 98 - protein, 494 aa, synthetic construct
  REGION 1..494: note = Description of Artificial Sequence: Synthetic polypeptide
DIQMTQSPSSLSASVGDRVTITCRSSTGAVTTSNYANWVQQKPGKAPKGLIGGTNKRAPGVPARFSGSGSGTDFTLTISSLQPEDFATYYCALWYSNLWVFGQGTKVEIKGGSGGSQVQLVQSGAEVKKPGASVKVSCKASGYTFTSYDINWVRQAPGQGLEWMGWMNPNSGNTGFAQKFQGRVTMTRDTSTSTVYMELSSLRSEDTAVYYCARDRANTDFSYGMDVWGQGTLVTVSSGGSGQSVLTQPPSASGTPGQRVTISCSGSRSNIGSNTVNWYQQLPGTAPKLLIYGNNQRPSGVPDRFSGSKSGTSASLAISGLQSEDEADYYCATWDDSLIGWVFGGGTKLTVLGGSGGSEVQLVESGGGLVQPGGSLRLSCAASGFTFSTYAMNWVRQAPGKGLEWVGRIRSKYNNYATYYADSVKDRFTISRDDSKNSLYLQMNSLKTEDTAVYYCARHGNFGNSYVSWFAYWGQGTLVTVSSAAAGSHHHHHH

SEQ ID NO: 99 - protein, 494 aa, synthetic construct
  REGION 1..494: note = Description of Artificial Sequence: Synthetic polypeptide
DIQMTQSPSSLSASVGDRVTITCRSSTGAVTTSNYANWVQQKPGKAPKGLIGGTNKRAPGVPARFSGSGSGTDFTLTISSLQPEDFATYYCALWYSNLWVFGQGTKVEIKGGSGGSQVQLVQSGAEVKKPGASVKVSCKASGYTFTSYDINWVRQAPGQGLEWMGWMNPNSGNTGFAQKFQGRVTMTRDTSTSTVYMELSSLRSEDTAVYYCARDRAVTDYYYGMDVWGQGTLVTVSSGGSGQSVLTQPPSASGTPGQRVTISCSGSRSNIGSNTVNWYQQLPGTAPKLLIYGNNQRPSGVPDRFSGSKSGTSASLAISGLQSEDEADYYCATWDDSLIGWVFGGGTKLTVLGGSGGSEVQLVESGGGLVQPGGSLRLSCAASGFTFSTYAMNWVRQAPGKGLEWVGRIRSKYNNYATYYADSVKDRFTISRDDSKNSLYLQMNSLKTEDTAVYYCARHGNFGNSYVSWFAYWGQGTLVTVSSAAAGSHHHHHH

SEQ ID NO: 100 - protein, 494 aa, synthetic construct
  REGION 1..494: note = Description of Artificial Sequence: Synthetic polypeptide
DIQMTQSPSSLSASVGDRVTITCRSSTGAVTTSNYANWVQQKPGKAPKGLIGGTNKRAPGVPARFSGSGSGTDFTLTISSLQPEDFATYYCALWYSNLWVFGQGTKVEIKGGSGGSQVQLVQSGAEVKKPGASVKVSCKASGYTFTSYDINWVRQAPGQGLEWMGWMNPNSGNTGFAQKFQGRVTMTRDTSTSTVYMELSSLRSEDTAVYYCARDRANTDYSFGMDVWGQGTLVTVSSGGSGQSVLTQPPSASGTPGQRVTISCSGSRSNIGSNTVNWYQQLPGTAPKLLIYGNNQRPSGVPDRFSGSKSGTSASLAISGLQSEDEADYYCATWDDSLIGWVFGGGTKLTVLGGSGGSEVQLVESGGGLVQPGGSLRLSCAASGFTFSTYAMNWVRQAPGKGLEWVGRIRSKYNNYATYYADSVKDRFTISRDDSKNSLYLQMNSLKTEDTAVYYCARHGNFGNSYVSWFAYWGQGTLVTVSSAAAGSHHHHHH

SEQ ID NO: 101 - protein, 494 aa, synthetic construct
  REGION 1..494: note = Description of Artificial Sequence: Synthetic polypeptide
DIQMTQSPSSLSASVGDRVTITCRSSTGAVTTSNYANWVQQKPGKAPKGLIGGTNKRAPGVPARFSGSGSGTDFTLTISSLQPEDFATYYCALWYSNLWVFGQGTKVEIKGGSGGSQVQLVQSGAEVKKPGASVKVSCKASGYTFTSYDINWVRQAPGQGLEWMGWMNPNSGNTGFAQKFQGRVTMTRDTSTSTVYMELSSLRSEDTAVYYCARDRANTDYSLGMDVWGQGTLVTVSSGGSGQSVLTQPPSASGTPGQRVTISCSGSRSNIGSNTVNWYQQLPGTAPKLLIYGNNQRPSGVPDRFSGSKSGTSASLAISGLQSEDEADYYCATWDDSLIGWVFGGGTKLTVLGGSGGSEVQLVESGGGLVQPGGSLRLSCAASGFTFSTYAMNWVRQAPGKGLEWVGRIRSKYNNYATYYADSVKDRFTISRDDSKNSLYLQMNSLKTEDTAVYYCARHGNFGNSYVSWFAYWGQGTLVTVSSAAAGSHHHHHH

SEQ ID NO: 102 - protein, 495 aa, synthetic construct
  REGION 1..495: note = Description of Artificial Sequence: Synthetic polypeptide
DIQMTQSPSSLSASVGDRVTITCRSSTGAVTTSNYANWVQQKPGKAPKGLIGGTNKRAPGVPARFSGSGSGTDFTLTISSLQPEDFATYYCALWYSNLWVFGQGTKVEIKGGSGGSQVQLVQSGAEVKKPGASVKVSCKASGYTFTSYDINWVRQAPGQGLEWMGWMNPNSGNTGFAQKFQGRVTMTRDTSTSTVYMELSSLRSEDTAVYYCARDRANTDYSFGMDVWGQGTLVTVSSGGSGGQSVLTQPPSASGTPGQRVTISCSGSRSNIGSNTVNWYQQLPGTAPKLLIYGNNQRPSGVPDRFSGSKSGTSASLAISGLQSEDEADYYCATWDDSLIGWVFGGGTKLTVLGGSGGSEVQLVESGGGLVQPGGSLRLSCAASGFTFSTYAMNWVRQAPGKGLEWVGRIRSKYNNYATYYADSVKDRFTISRDDSKNSLYLQMNSLKTEDTAVYYCARHGNFGNSYVSWFAYWGQGTLVTVSSAAAGSHHHHHH

SEQ ID NO: 103 - protein, 495 aa, synthetic construct
  REGION 1..495: note = Description of Artificial Sequence: Synthetic polypeptide
DIQMTQSPSSLSASVGDRVTITCRSSTGAVTTSNYANWVQQKPGKAPKGLIGGTNKRAPGVPARFSGSGSGTDFTLTISSLQPEDFATYYCALWYSNLWVFGQGTKVEIKGGSGGSQVQLVQSGAEVKKPGASVKVSCKASGYTFTSYDINWVRQAPGQGLEWMGWMNPNSGNTGFAQKFQGRVTMTRDTSTSTVYMELSSLRSEDTAVYYCARDRANTDYSLGMDVWGQGTLVTVSSGGSGGQSVLTQPPSASGTPGQRVTISCSGSRSNIGSNTVNWYQQLPGTAPKLLIYGNNQRPSGVPDRFSGSKSGTSASLAISGLQSEDEADYYCATWDDSLIGWVFGGGTKLTVLGGSGGSEVQLVESGGGLVQPGGSLRLSCAASGFTFSTYAMNWVRQAPGKGLEWVGRIRSKYNNYATYYADSVKDRFTISRDDSKNSLYLQMNSLKTEDTAVYYCARHGNFGNSYVSWFAYWGQGTLVTVSSAAAGSHHHHHH

SEQ ID NO: 104 - protein, 491 aa, synthetic construct
  REGION 1..491: note = Description of Artificial Sequence: Synthetic polypeptide
DIQMTQSPSSLSASVGDRVTITCRSSTGAVTTSNYANWVQQKPGKAPKALIGGTNKRAPGVPSRFSGSLIGDKATLTISSLQPEDFATYYCALWYSNLWVFGQGTKVEIKGGSGGSQVQLQESGGGVVQPGRSLRLSCAASGFSFSNYGIHWVRQAPGKGLEWVALISYDGNKKFYADSVKGRFAISRDTSKNTVDLQMTSLRPEDTAVYYCAKDRLESAAFDYWGQGTLVTVSSGGSGGSSYELTQPPSVSVAPGQTAMITCGGNNIGSTTVHWYQQKPGQAPVLVVYDDNERPSGIPERFSGSNSGSTATLTINRVEAGDEADYYCQVWDSGSDHVVFGGGTKLTVLGGSGGSEVQLVESGGGLVQPGGSLRLSCAASGFTFSTYAMNWVRQAPGKGLEWVGRIRSKYNNYATYYADSVKDRFTISRDDSKNSLYLQMNSLKTEDTAVYYCARHGNFGNSYVSYFAYWGQGTLVTVSSAAAGSHHHHHH

SEQ ID NO: 105 - protein, 496 aa, synthetic construct
  REGION 1..496: note = Description of Artificial Sequence: Synthetic polypeptide
QSVLTQPPSASGTPGQRVTISCSGSRSNIGSNTVNWYQQLPGTAPKLLIYGNNQRPSGVPDRFSGSKSGTSASLAISGLQSEDEADYYCATWDDSLIGWVFGGGTKLTVLGGSGGSEVQLVESGGGLVQPGGSLRLSCAASGFTFSTYAMNWVRQAPGKGLEWVGRIRSKYNNYATYYADSVKDRFTISRDDSKNSLYLQMNSLKTEDTAVYYCARHGNFGNSYVSYFAYWGQGTLVTVSSGGSGGSDIQMTQSPSSLSASVGDRVTITCRSSTGAVTTSNYANWVQQKPGKAPKALIGGTNKRAPGVPSRFSGSLIGDKATLTISSLQPEDFATYYCALWYSNLWVFGQGTKVEIKGGSGGSQVQLVQSGAEVKKPGASVKVSCKASGYTFTSYDINWVRQAPGQGLEWMGWMNPNSGNTGFAQKFQGRVTMTRDTSTSTVYMELSSLRSEDTAVYYCARDRANTDFSYGMDVWGQGTLVTVSSAAAGSHHHHHH

SEQ ID NO: 106 - protein, 494 aa, synthetic construct
  REGION 1..494: note = Description of Artificial Sequence: Synthetic polypeptide
DIQMTQSPSSLSASVGDRVTITCRSSTGAVTTSNYANWVQQKPGKAPKGLIGGTNKRAPGVPSRFSGSLIGDKATLTISSLQPEDFATYYCALWYSNLWVFGQGTKVEIKGGSGGSQVQLVQSGAEVKKPGASVKVSCKASGYTFTSYDINWVRQAPGQGLEWMGWMNPNSGNTGFAQKFQGRVTMTRDTSTSTVYMELSSLRSEDTAVYYCARDRANTDFSYGMDVWGQGTLVTVSSGGSGQSVLTQPPSASGTPGQRVTISCSGSRSNIGSNTVNWYQQLPGTAPKLLIYGNNQRPSGVPDRFSGSKSGTSASLAISGLQSEDEADYYCATWDDSLIGWVFGGGTKLTVLGGSGGSEVQLVESGGGLVQPGGSLRLSCAASGFTFSTYAMNWVRQAPGKGLEWVGRIRSKYNNYATYYADSVKDRFTISRDDSKNSLYLQMNSLKTEDTAVYYCARHGNFGNSYVSWFAYWGQGTLVTVSSAAAGSHHHHHH

SEQ ID NO: 107 - protein, 494 aa, synthetic construct
  REGION 1..494: note = Description of Artificial Sequence: Synthetic polypeptide
DIQMTQSPSSLSASVGDRVTITCRSSTGAVTTSNYANWVQQKPGKAPKGLIGGTNKRAPGVPSRFSGSLIGDKATLTISSLQPEDFATYYCALWYSNLWVFGQGTKVEIKGGSGGSQVQLVQSGAEVKKPGASVKVSCKASGYTFTSYDINWVRQAPGQGLEWMGWMNPNSGNTGFAQKFQGRVTMTRDTSTSTVYMELSSLRSEDTAVYYCARDRANTDYSFGMDVWGQGTLVTVSSGGSGQSVLTQPPSASGTPGQRVTISCSGSRSNIGSNTVNWYQQLPGTAPKLLIYGNNQRPSGVPDRFSGSKSGTSASLAISGLQSEDEADYYCATWDDSLIGWVFGGGTKLTVLGGSGGSEVQLVESGGGLVQPGGSLRLSCAASGFTFSTYAMNWVRQAPGKGLEWVGRIRSKYNNYATYYADSVKDRFTISRDDSKNSLYLQMNSLKTEDTAVYYCARHGNFGNSYVSWFAYWGQGTLVTVSSAAAGSHHHHHH

SEQ ID NO: 108 - protein, 494 aa, synthetic construct
  REGION 1..494: note = Description of Artificial Sequence: Synthetic polypeptide
DIQMTQSPSSLSASVGDRVTITCRSSTGAVTTSNYANWVQQKPGKAPKGLIGGTNKRAPGVPSRFSGSLIGDKATLTISSLQPEDFATYYCALWYSNLWVFGQGTKVEIKGGSGGSQVQLVQSGAEVKKPGASVKVSCKASGYTFTSYDINWVRQAPGQGLEWMGWMNPNSGNTGFAQKFQGRVTMTRDTSTSTVYMELSSLRSEDTAVYYCARDRANTDYSLGMDVWGQGTLVTVSSGGSGQSVLTQPPSASGTPGQRVTISCSGSRSNIGSNTVNWYQQLPGTAPKLLIYGNNQRPSGVPDRFSGSKSGTSASLAISGLQSEDEADYYCATWDDSLIGWVFGGGTKLTVLGGSGGSEVQLVESGGGLVQPGGSLRLSCAASGFTFSTYAMNWVRQAPGKGLEWVGRIRSKYNNYATYYADSVKDRFTISRDDSKNSLYLQMNSLKTEDTAVYYCARHGNFGNSYVSWFAYWGQGTLVTVSSAAAGSHHHHHH

SEQ ID NO: 109 - protein, 494 aa, synthetic construct
  REGION 1..494: note = Description of Artificial Sequence: Synthetic polypeptide
DIQMTQSPSSLSASVGDRVTITCRSSTGAVTTSNYANWVQQKPGKAPKALIGGTNKRAPGVPSRFSGSLIGDKATLTISSLQPEDFATYYCALWYSNLWVFGQGTKVEIKGGSGGSQVQLVQSGAEVKKPGASVKVSCKASGYTFTSYDINWVRQAPGQGLEWMGWMNPNSGNTGFAQKFQGRVTMTRDTSTSTVYMELSSLRSEDTAVYYCARDRAVTDYYYGMDVWGQGTLVTVSSGGSGQSVLTQPPSASGTPGQRVTISCSGSRSNIGSNTVNWYQQLPGTAPKLLIYGNNQRPSGVPDRFSGSKSGTSASLAISGLQSEDEADYYCATWDDSLIGWVFGGGTKLTVLGGSGGSEVQLVESGGGLVQPGGSLRLSCAASGFTFSTYAMNWVRQAPGKGLEWVGRIRSKYNNYATYYADSVKDRFTISRDDSKNSLYLQMNSLKTEDTAVYYCARHGNFGNSYVSYFAYWGQGTLVTVSSAAAGSHHHHHH

SEQ ID NO: 110 - protein, 494 aa, synthetic construct
  REGION 1..494: note = Description of Artificial Sequence: Synthetic polypeptide
DIQMTQSPSSLSASVGDRVTITCRSSTGAVTTSNYANWVQQKPGKAPKGLIGGTNKRAPGVPSRFSGSLIGTDFTLTISSLQPEDFATYYCALWYSNLWVFGQGTKVEIKGGSGGSQVQLVQSGAEVKKPGASVKVSCKASGYTFTSYDINWVRQAPGQGLEWMGWMNPNSGNTGFAQKFQGRVTMTRDTSTSTVYMELSSLRSEDTAVYYCARDRAVTDYYYGMDVWGQGTLVTVSSGGSGQSVLTQPPSASGTPGQRVTISCSGSRSNIGSNTVNWYQQLPGTAPKLLIYGNNQRPSGVPDRFSGSKSGTSASLAISGLQSEDEADYYCATWDDSLIGWVFGGGTKLTVLGGSGGSEVQLVESGGGLVQPGGSLRLSCAASGFTFSTYAMNWVRQAPGKGLEWVGRIRSKYNNYATYYADSVKDRFTISRDDSKNSLYLQMNSLKTEDTAVYYCARHGNFGNSYVSWFAYWGQGTLVTVSSAAAGSHHHHHH

SEQ ID NO: 111 - protein, 494 aa, synthetic construct
  REGION 1..494: note = Description of Artificial Sequence: Synthetic polypeptide
DIQMTQSPSSLSASVGDRVTITCRSSTGAVTTSNYANWVQQKPGKAPKALIGGTNKRAPGVPSRFSGSLIGDKATLTISSLQPEDFATYYCALWYSNLWVFGQGTKVEIKGGSGGSQVQLVQSGAEVKKPGASVKVSCKASGYTFTSYDINWVRQAPGQGLEWMGWMNPNSGNTGFAQKFQGRVTMTRDTSTSTVYMELSSLRSEDTAVYYCARDRANTDFSYGMDVWGQGTLVTVSSGGSGQSVLTQPPSASGTPGQRVTISCSGSRSNIGSNTVNWYQQLPGTAPKLLIYGNNQRPSGVPDRFSGSKSGSSASLAISGLQSEDEADYYCATWDDSLIGWVFGGGTKLTVLGGSGGSEVQLVESGGGLVQPGGSLRLSCAASGFTFSTYAMNWVRQAPGKGLEWVGRIRSKYNNYATYYADSVKDRFTISRDDSKNSLYLQMNSLKTEDTAVYYCARHGNFGNSYVSYFAYWGQGTLVTVSSAAAGSHHHHHH

SEQ ID NO: 112 - protein, 494 aa, synthetic construct
  REGION 1..494: note = Description of Artificial Sequence: Synthetic polypeptide
DIQMTQSPSSLSASVGDRVTITCRSSTGAVTTSNYANWVQQKPGKAPKALIGGTNKRAPGVPSRFSGSLIGDKATLTISSLQPEDFATYYCALWYSNLWVFGQGTKVEIKGGSGGSQVQLVQSGAEVKKPGASVKVSCKASGYTFTSYDINWVRQAPGQGLEWMGWMNPNSGNTGFAQKFQGRVTMTRDTSTSTVYMELSSLRSEDTAVYYCARDRANTDYSFGMDVWGQGTLVTVSSGGSGQSVLTQPPSASGTPGQRVTISCSGSRSNIGSNTVNWYQQLPGTAPKLLIYGNNQRPSGVPDRFSGSKSGTSASLAISGLQSEDEADYYCATWDDSLIGWVFGGGTKLTVLGGSGGSEVQLVESGGGLVQPGGSLRLSCAASGFTFSTYAMNWVRQAPGKGLEWVGRIRSKYNNYATYYADSVKDRFTISRDDSKNSLYLQMNSLKTEDTAVYYCARHGNFGNSYVSYFAYWGQGTLVTVSSAAAGSHHHHHH

SEQ ID NO: 113 - protein, 494 aa, synthetic construct
  REGION 1..494: note = Description of Artificial Sequence: Synthetic polypeptide
DIQMTQSPSSLSASVGDRVTITCRSSTGAVTTSNYANWVQQKPGKAPKALIGGTNKRAPGVPSRFSGSLIGDKATLTISSLQPEDFATYYCALWYSNLWVFGQGTKVEIKGGSGGSQVQLVQSGAEVKKPGASVKVSCKASGYTFTSYDINWVRQAPGQGLEWMGWMNPNSGNTGFAQKFQGRVTMTRDTSTSTVYMELSSLRSEDTAVYYCARDRANTDYSLGMDVWGQGTLVTVSSGGSGQSVLTQPPSASGTPGQRVTISCSGSRSNIGSNTVNWYQQLPGTAPKLLIYGNNQRPSGVPDRFSGSKSGTSASLAISGLQSEDEADYYCATWDDSLIGWVFGGGTKLTVLGGSGGSEVQLVESGGGLVQPGGSLRLSCAASGFTFSTYAMNWVRQAPGKGLEWVGRIRSKYNNYATYYADSVKDRFTISRDDSKNSLYLQMNSLKTEDTAVYYCARHGNFGNSYVSYFAYWGQGTLVTVSSAAAGSHHHHHH

SEQ ID NO: 114 - protein, 492 aa, synthetic construct
  REGION 1..492: note = Description of Artificial Sequence: Synthetic polypeptide
DIQMTQSPSSLSASVGDRVTITCRSSTGAVTTSNYANWVQQKPGKAPKALIGGTNKRAPGVPSRFSGSLIGDKATLTISSLQPEDFATYYCALWYSNLWVFGQGTKVEIKGGSGGSQVQLVQSGAEVKKPGESLKISCKGSGYSFTSYWIGWVRQMPGKGLEWMGIIYPGDSDTRYSPSFQGQVTISADKSISTAYLQWSSLKASDTAMYYCARHKRGSDAFDIWGQGTTVTVSSGGSGQSVLTQPPSVSGAPGQRVTISCTGSSSNIGAGYDVHWYQQLPGTAPKLLIYGNSNRPSGVPDRFSGSKSGTSASLAITGLQAEDEADYYCQSYDSSLSDVVFGGGTKLTVLGGSGGSEVQLVESGGGLVQPGGSLRLSCAASGFTFSTYAMNWVRQAPGKGLEWVGRIRSKYNNYATYYADSVKDRFTISRDDSKNSLYLQMNSLKTEDTAVYYCARHGNFGNSYVSYFAYWGQGTLVTVSSAAAGSHHHHHH

SEQ ID NO: 115 - protein, 492 aa, synthetic construct
  REGION 1..492: note = Description of Artificial Sequence: Synthetic polypeptide
EVQLVESGGGLVQPGGSLRLSCAASGFTFSTYAMNWVRQAPGKGLEWVGRIRSKYNNYATYYADSVKDRFTISRDDSKNSLYLQMNSLKTEDTAVYYCARHGNFGNSYVSYFAYWGQGTLVTVSSGGSGGSQSVLTQPPSVSGAPGQRVTISCTGSSSNIGAGYDVHWYQQLPGTAPKLLIYGNSNRPSGVPDRFSGSKSGTSASLAITGLQAEDEADYYCQSYDSSLSDVVFGGGTKLTVLGGSGQVQLVQSGAEVKKPGESLKISCKGSGYSFTSYWIGWVRQMPGKGLEWMGIIYPGDSDTRYSPSFQGQVTISADKSISTAYLQWSSLKASDTAMYYCARHKRGSDAFDIWGQGTTVTVSSGGSGGSDIQMTQSPSSLSASVGDRVTITCRSSTGAVTTSNYANWVQQKPGKAPKALIGGTNKRAPGVPSRFSGSLIGDKATLTISSLQPEDFATYYCALWYSNLWVFGQGTKVEIKAAAGSHHHHHH

SEQ ID NO: 116 - protein, 495 aa, synthetic construct
  REGION 1..495: note = Description of Artificial Sequence: Synthetic polypeptide
DIQMTQSPSSLSASVGDRVTITCRSSTGAVTTSNYANWVQQKPGKAPKALIGGTNKRAPGVPSRFSGSLIGDKATLTISSLQPEDFATYYCALWYSNLWVFGQGTKVEIKGGSGGSQVQLVQSGAEVKKPGASVKVSCKASGYTFTSYYMHWVRQAPGQGLEWMGIINPSGGSTSYAQKFQGRVTMTRDTSTSTVYMELSSLRSEDTAVYYCARDVVPAAIDYYGMDVWGQGTTVTVSSGGSGQSVLTQPPSASGTPGQRVTISCSGSSSNIGSNTVNWYQQLPGTAPKLLIYSDNQRPSGVPDRFSGSKSGSSASLAISGLQSDDEADYYCATWDDSLNGAVFGGGTKLTVLGGSGGSEVQLVESGGGLVQPGGSLRLSCAASGFTFSTYAMNWVRQAPGKGLEWVGRIRSKYNNYATYYADSVKDRFTISRDDSKNSLYLQMNSLKTEDTAVYYCARHGNFGNSYVSYFAYWGQGTLVTVSSAAAGSHHHHHH

SEQ ID NO: 117 - protein, 495 aa, synthetic construct
  REGION 1..495: note = Description of Artificial Sequence: Synthetic polypeptide
DIQMTQSPSSLSASVGDRVTITCRSSTGAVTTSNYANWVQQKPGKAPKGLIGGTNKRAPGVPSRFSGSLIGTDFTLTISSLQPEDFATYYCALWYSNLWVFGQGTKVEIKGGSGGSQVQLVQSGAEVKKPGASVKVSCKASGYTFTSYYMHWVRQAPGQGLEWMGIINPSGGSTSYAQKFQGRVTMTRDTSTSTVYMELSSLRSEDTAVYYCARDVVPAAIDYYGMDVWGQGTTVTVSSGGSGQSVLTQPPSASGTPGQRVTISCSGSSSNIGSNTVNWYQQLPGTAPKLLIYSDNQRPSGVPDRFSGSKSGSSASLAISGLQSDDEADYYCATWDDSLNGAVFGGGTKLTVLGGSGGSEVQLVESGGGLVQPGGSLRLSCAASGFTFSTYAMNWVRQAPGKGLEWVGRIRSKYNNYATYYADSVKDRFTISRDDSKNSLYLQMNSLKTEDTAVYYCARHGNFGNSYVSWFAYWGQGTLVTVSSAAAGSHHHHHH

SEQ ID NO: 118 - protein, 494 aa, synthetic construct
  REGION 1..494: note = Description of Artificial Sequence: Synthetic polypeptide
DIQMTQSPSSLSASVGDRVTITCRSSTGAVTTSNYANWVQQKPGKAPKALIGGTNKRAPGVPSRFSGSLIGDKATLTISSLQPEDFATYYCALWYSNLWVFGQGTKVEIKGGSGGSQVQLVQSGAEVKKPGSSVKVSCKASGGTFSSYAISWVRQAPGQGLEWMGGIYPIFGSANYAQKFQGRVTITADESTSTAYMELSSLRSEDTAVYYCAREYYYDSSEWAFDIWGQGTLVTVSSGGSGQSVLTQPPSASGTPGQRVTISCSGSSSNIGSNIVNWYQQLPGTAPKLLIYSNNQRPSGVPDRFSGSKSGTSASLAISGLQSEDEADYYCAAWDDSLKGYVFGGGTKLTVLGGSGGSEVQLVESGGGLVQPGGSLRLSCAASGFTFSTYAMNWVRQAPGKGLEWVGRIRSKYNNYATYYADSVKDRFTISRDDSKNSLYLQMNSLKTEDTAVYYCARHGNFGNSYVSYFAYWGQGTLVTVSSAAAGSHHHHHH

SEQ ID NO: 119 - protein, 494 aa, synthetic construct
  REGION 1..494: note = Description of Artificial Sequence: Synthetic polypeptide
DIQMTQSPSSLSASVGDRVTITCRSSTGAVTTSNYANWVQQKPGKAPKALIGGTNKRAPGVPSRFSGSLIGDKATLTISSLQPEDFATYYCALWYSNLWVFGQGTKVEIKGGSGGSQVQLVQSGAEVKKPGSSVKVSCKASGGTFSSYGISWVRQAPGQGLEWMGGIIPIFGSAHYAQKFQGRVTITADESTSTAYMELSSLRSEDTAVYYCAREYYYDSSEWAFDIWGQGTLVTVSSGGSGQSVLTQPPSASGTPGQRVTISCSGSSSNIGSNTVKWYQQLPGTAPKLLIYSNNQRSSGVPDRFSGSKSGTSASLAISGLQSEDEADYYCAAWDDSLNGYVFGGGTKLTVLGGSGGSEVQLVESGGGLVQPGGSLRLSCAASGFTFSTYAMNWVRQAPGKGLEWVGRIRSKYNNYATYYADSVKDRFTISRDDSKNSLYLQMNSLKTEDTAVYYCARHGNFGNSYVSYFAYWGQGTLVTVSSAAAGSHHHHHH

SEQ ID NO: 120 - protein, 494 aa, synthetic construct
  REGION 1..494: note = Description of Artificial Sequence: Synthetic polypeptide
DIQMTQSPSSLSASVGDRVTITCRSSTGAVTTSNYANWVQQKPGKAPKGLIGGTNKRAPGVPSRFSGSLIGTDFTLTISSLQPEDFATYYCALWYSNLWVFGQGTKVEIKGGSGGSQVQLVQSGAEVKKPGSSVKVSCKASGGTFSSYGISWVRQAPGQGLEWMGGIIPIFGSAHYAQKFQGRVTITADESTSTAYMELSSLRSEDTAVYYCAREYYYDSSEWAFDIWGQGTLVTVSSGGSGQSVLTQPPSASGTPGQRVTISCSGSSSNIGSNTVKWYQQLPGTAPKLLIYSNNQRSSGVPDRFSGSKSGTSASLAISGLQSEDEADYYCAAWDDSLNGYVFGGGTKLTVLGGSGGSEVQLVESGGGLVQPGGSLRLSCAASGFTFSTYAMNWVRQAPGKGLEWVGRIRSKYNNYATYYADSVKDRFTISRDDSKNSLYLQMNSLKTEDTAVYYCARHGNFGNSYVSWFAYWGQGTLVTVSSAAAGSHHHHHH

SEQ ID NO: 121 - protein, 494 aa, synthetic construct
  REGION 1..494: note = Description of Artificial Sequence: Synthetic polypeptide
DIQMTQSPSSLSASVGDRVTITCRSSTGAVTTSNYANWVQQKPGKAPKALIGGTNKRAPGVPSRFSGSLIGDKATLTISSLQPEDFATYYCALWYSNLWVFGQGTKVEIKGGSGGSQVQLVQSGAEVKKPGSSVKVSCKASGGTFDSYAISWVRQAPGQGLEWMGGIIPIFGSAHYSQKFQGRVTITADESTSTAYMELSSLRSEDTAVYYCAREYYYDSSEWAFDIWGQGTLVTVSSGGSGQSVLTQPPSASGTPGQRVTISCSGSSSNIGDNVVNWYQQLPGTAPKLLIYSTNKRPSGVPDRFSGSKSGSSASLAISGLQSEDEADYYCAAWDDSLSAYVFGGGTKLTVLGGSGGSEVQLVESGGGLVQPGGSLRLSCAASGFTFSTYAMNWVRQAPGKGLEWVGRIRSKYNNYATYYADSVKDRFTISRDDSKNSLYLQMNSLKTEDTAVYYCARHGNFGNSYVSYFAYWGQGTLVTVSSAAAGSHHHHHH

SEQ ID NO: 122 - protein, 6 aa, synthetic construct
  REGION 1..6: note = Description of Artificial Sequence: Synthetic 6xHis tag
HHHHHH

SEQ ID NO: 123 - protein, 483 aa, synthetic construct
  REGION 1..483: note = Synthetic polypeptide
DIQMTQSPSSLSASVGDRVTITCRSSTGAVTTSNYANWVQQKPGKAPKGLIGGTNKRAPGVPARFSGSGSGTDFTLTISSLQPEDFATYYCALWYSNLWVFGQGTKVEIKGGSGGSQVQLVQSGAEVKKPGASVKVSCKASGYTFTSYDINWVRQAPGQGLEWMGWMNPNSGNTGFAQKFQGRVTMTRDTSTSTVYMELSSLRSEDTAVYYCARDRANTDFSYGMDVWGQGTLVTVSSGGSGQSVLTQPPSASGTPGQRVTISCSGSRSNIGSNTVNWYQQLPGTAPKLLIYGNNQRPSGVPDRFSGSKSGTSASLAISGLQSEDEADYYCATWDDSLIGWVFGGGTKLTVLGGSGGSEVQLVESGGGLVQPGGSLRLSCAASGFTFSTYAMNWVRQAPGKGLEWVGRIRSKYNNYATYYADSVKDRFTISRDDSKNSLYLQMNSLKTEDTAVYYCARHGNFGNSYVSWFAYWGQGTLVTVSS

SEQ ID NO: 124 - protein, 483 aa, synthetic construct
  REGION 1..483: note = Synthetic polypeptide
DIQMTQSPSSLSASVGDRVTITCRSSTGAVTTSNYANWVQQKPGKAPKGLIGGTNKRAPGVPARFSGSGSGTDFTLTISSLQPEDFATYYCALWYSNLWVFGQGTKVEIKGGSGGSQVQLVQSGAEVKKPGASVKVSCKASGYTFTSYDINWVRQAPGQGLEWMGWMNPNSGNTGFAQKFQGRVTMTRDTSTSTVYMELSSLRSEDTAVYYCARDRAVTDYYYGMDVWGQGTLVTVSSGGSGQSVLTQPPSASGTPGQRVTISCSGSRSNIGSNTVNWYQQLPGTAPKLLIYGNNQRPSGVPDRFSGSKSGTSASLAISGLQSEDEADYYCATWDDSLIGWVFGGGTKLTVLGGSGGSEVQLVESGGGLVQPGGSLRLSCAASGFTFSTYAMNWVRQAPGKGLEWVGRIRSKYNNYATYYADSVKDRFTISRDDSKNSLYLQMNSLKTEDTAVYYCARHGNFGNSYVSWFAYWGQGTLVTVSS

SEQ ID NO: 125 - protein, 483 aa, synthetic construct
  REGION 1..483: note = Synthetic polypeptide
DIQMTQSPSSLSASVGDRVTITCRSSTGAVTTSNYANWVQQKPGKAPKGLIGGTNKRAPGVPARFSGSGSGTDFTLTISSLQPEDFATYYCALWYSNLWVFGQGTKVEIKGGSGGSQVQLVQSGAEVKKPGASVKVSCKASGYTFTSYDINWVRQAPGQGLEWMGWMNPNSGNTGFAQKFQGRVTMTRDTSTSTVYMELSSLRSEDTAVYYCARDRANTDYSFGMDVWGQGTLVTVSSGGSGQSVLTQPPSASGTPGQRVTISCSGSRSNIGSNTVNWYQQLPGTAPKLLIYGNNQRPSGVPDRFSGSKSGTSASLAISGLQSEDEADYYCATWDDSLIGWVFGGGTKLTVLGGSGGSEVQLVESGGGLVQPGGSLRLSCAASGFTFSTYAMNWVRQAPGKGLEWVGRIRSKYNNYATYYADSVKDRFTISRDDSKNSLYLQMNSLKTEDTAVYYCARHGNFGNSYVSWFAYWGQGTLVTVSS

SEQ ID NO: 126 - protein, 483 aa, synthetic construct
  REGION 1..483: note = Synthetic polypeptide
DIQMTQSPSSLSASVGDRVTITCRSSTGAVTTSNYANWVQQKPGKAPKGLIGGTNKRAPGVPARFSGSGSGTDFTLTISSLQPEDFATYYCALWYSNLWVFGQGTKVEIKGGSGGSQVQLVQSGAEVKKPGASVKVSCKASGYTFTSYDINWVRQAPGQGLEWMGWMNPNSGNTGFAQKFQGRVTMTRDTSTSTVYMELSSLRSEDTAVYYCARDRANTDYSLGMDVWGQGTLVTVSSGGSGQSVLTQPPSASGTPGQRVTISCSGSRSNIGSNTVNWYQQLPGTAPKLLIYGNNQRPSGVPDRFSGSKSGTSASLAISGLQSEDEADYYCATWDDSLIGWVFGGGTKLTVLGGSGGSEVQLVESGGGLVQPGGSLRLSCAASGFTFSTYAMNWVRQAPGKGLEWVGRIRSKYNNYATYYADSVKDRFTISRDDSKNSLYLQMNSLKTEDTAVYYCARHGNFGNSYVSWFAYWGQGTLVTVSS

SEQ ID NO: 127 - protein, 484 aa, synthetic construct
  REGION 1..484: note = Synthetic polypeptide
DIQMTQSPSSLSASVGDRVTITCRSSTGAVTTSNYANWVQQKPGKAPKGLIGGTNKRAPGVPARFSGSGSGTDFTLTISSLQPEDFATYYCALWYSNLWVFGQGTKVEIKGGSGGSQVQLVQSGAEVKKPGASVKVSCKASGYTFTSYDINWVRQAPGQGLEWMGWMNPNSGNTGFAQKFQGRVTMTRDTSTSTVYMELSSLRSEDTAVYYCARDRANTDYSFGMDVWGQGTLVTVSSGGSGGQSVLTQPPSASGTPGQRVTISCSGSRSNIGSNTVNWYQQLPGTAPKLLIYGNNQRPSGVPDRFSGSKSGTSASLAISGLQSEDEADYYCATWDDSLIGWVFGGGTKLTVLGGSGGSEVQLVESGGGLVQPGGSLRLSCAASGFTFSTYAMNWVRQAPGKGLEWVGRIRSKYNNYATYYADSVKDRFTISRDDSKNSLYLQMNSLKTEDTAVYYCARHGNFGNSYVSWFAYWGQGTLVTVSS

SEQ ID NO: 128 - protein, 484 aa, synthetic construct
  REGION 1..484: note = Synthetic polypeptide
DIQMTQSPSSLSASVGDRVTITCRSSTGAVTTSNYANWVQQKPGKAPKGLIGGTNKRAPGVPARFSGSGSGTDFTLTISSLQPEDFATYYCALWYSNLWVFGQGTKVEIKGGSGGSQVQLVQSGAEVKKPGASVKVSCKASGYTFTSYDINWVRQAPGQGLEWMGWMNPNSGNTGFAQKFQGRVTMTRDTSTSTVYMELSSLRSEDTAVYYCARDRANTDYSLGMDVWGQGTLVTVSSGGSGGQSVLTQPPSASGTPGQRVTISCSGSRSNIGSNTVNWYQQLPGTAPKLLIYGNNQRPSGVPDRFSGSKSGTSASLAISGLQSEDEADYYCATWDDSLIGWVFGGGTKLTVLGGSGGSEVQLVESGGGLVQPGGSLRLSCAASGFTFSTYAMNWVRQAPGKGLEWVGRIRSKYNNYATYYADSVKDRFTISRDDSKNSLYLQMNSLKTEDTAVYYCARHGNFGNSYVSWFAYWGQGTLVTVSS

SEQ ID NO: 129 - protein, 480 aa, synthetic construct
  REGION 1..480: note = Synthetic polypeptide
DIQMTQSPSSLSASVGDRVTITCRSSTGAVTTSNYANWVQQKPGKAPKALIGGTNKRAPGVPSRFSGSLIGDKATLTISSLQPEDFATYYCALWYSNLWVFGQGTKVEIKGGSGGSQVQLQESGGGVVQPGRSLRLSCAASGFSFSNYGIHWVRQAPGKGLEWVALISYDGNKKFYADSVKGRFAISRDTSKNTVDLQMTSLRPEDTAVYYCAKDRLESAAFDYWGQGTLVTVSSGGSGGSSYELTQPPSVSVAPGQTAMITCGGNNIGSTTVHWYQQKPGQAPVLVVYDDNERPSGIPERFSGSNSGSTATLTINRVEAGDEADYYCQVWDSGSDHVVFGGGTKLTVLGGSGGSEVQLVESGGGLVQPGGSLRLSCAASGFTFSTYAMNWVRQAPGKGLEWVGRIRSKYNNYATYYADSVKDRFTISRDDSKNSLYLQMNSLKTEDTAVYYCARHGNFGNSYVSYFAYWGQGTLVTVSS

SEQ ID NO: 130 - protein, 485 aa, synthetic construct
  REGION 1..485: note = Synthetic polypeptide
QSVLTQPPSASGTPGQRVTISCSGSRSNIGSNTVNWYQQLPGTAPKLLIYGNNQRPSGVPDRFSGSKSGTSASLAISGLQSEDEADYYCATWDDSLIGWVFGGGTKLTVLGGSGGSEVQLVESGGGLVQPGGSLRLSCAASGFTFSTYAMNWVRQAPGKGLEWVGRIRSKYNNYATYYADSVKDRFTISRDDSKNSLYLQMNSLKTEDTAVYYCARHGNFGNSYVSYFAYWGQGTLVTVSSGGSGGSDIQMTQSPSSLSASVGDRVTITCRSSTGAVTTSNYANWVQQKPGKAPKALIGGTNKRAPGVPSRFSGSLIGDKATLTISSLQPEDFATYYCALWYSNLWVFGQGTKVEIKGGSGGSQVQLVQSGAEVKKPGASVKVSCKASGYTFTSYDINWVRQAPGQGLEWMGWMNPNSGNTGFAQKFQGRVTMTRDTSTSTVYMELSSLRSEDTAVYYCARDRANTDFSYGMDVWGQGTLVTVSS

SEQ ID NO: 131 - protein, 483 aa, synthetic construct
  REGION 1..483: note = Synthetic polypeptide
DIQMTQSPSSLSASVGDRVTITCRSSTGAVTTSNYANWVQQKPGKAPKGLIGGTNKRAPGVPSRFSGSLIGDKATLTISSLQPEDFATYYCALWYSNLWVFGQGTKVEIKGGSGGSQVQLVQSGAEVKKPGASVKVSCKASGYTFTSYDINWVRQAPGQGLEWMGWMNPNSGNTGFAQKFQGRVTMTRDTSTSTVYMELSSLRSEDTAVYYCARDRANTDFSYGMDVWGQGTLVTVSSGGSGQSVLTQPPSASGTPGQRVTISCSGSRSNIGSNTVNWYQQLPGTAPKLLIYGNNQRPSGVPDRFSGSKSGTSASLAISGLQSEDEADYYCATWDDSLIGWVFGGGTKLTVLGGSGGSEVQLVESGGGLVQPGGSLRLSCAASGFTFSTYAMNWVRQAPGKGLEWVGRIRSKYNNYATYYADSVKDRFTISRDDSKNSLYLQMNSLKTEDTAVYYCARHGNFGNSYVSWFAYWGQGTLVTVSS

SEQ ID NO: 132 - protein, 483 aa, synthetic construct
  REGION 1..483: note = Synthetic polypeptide
DIQMTQSPSSLSASVGDRVTITCRSSTGAVTTSNYANWVQQKPGKAPKGLIGGTNKRAPGVPSRFSGSLIGDKATLTISSLQPEDFATYYCALWYSNLWVFGQGTKVEIKGGSGGSQVQLVQSGAEVKKPGASVKVSCKASGYTFTSYDINWVRQAPGQGLEWMGWMNPNSGNTGFAQKFQGRVTMTRDTSTSTVYMELSSLRSEDTAVYYCARDRANTDYSFGMDVWGQGTLVTVSSGGSGQSVLTQPPSASGTPGQRVTISCSGSRSNIGSNTVNWYQQLPGTAPKLLIYGNNQRPSGVPDRFSGSKSGTSASLAISGLQSEDEADYYCATWDDSLIGWVFGGGTKLTVLGGSGGSEVQLVESGGGLVQPGGSLRLSCAASGFTFSTYAMNWVRQAPGKGLEWVGRIRSKYNNYATYYADSVKDRFTISRDDSKNSLYLQMNSLKTEDTAVYYCARHGNFGNSYVSWFAYWGQGTLVTVSS

SEQ ID NO: 133 - protein, 483 aa, synthetic construct
  REGION 1..483: note = Synthetic polypeptide
DIQMTQSPSSLSASVGDRVTITCRSSTGAVTTSNYANWVQQKPGKAPKGLIGGTNKRAPGVPSRFSGSLIGDKATLTISSLQPEDFATYYCALWYSNLWVFGQGTKVEIKGGSGGSQVQLVQSGAEVKKPGASVKVSCKASGYTFTSYDINWVRQAPGQGLEWMGWMNPNSGNTGFAQKFQGRVTMTRDTSTSTVYMELSSLRSEDTAVYYCARDRANTDYSLGMDVWGQGTLVTVSSGGSGQSVLTQPPSASGTPGQRVTISCSGSRSNIGSNTVNWYQQLPGTAPKLLIYGNNQRPSGVPDRFSGSKSGTSASLAISGLQSEDEADYYCATWDDSLIGWVFGGGTKLTVLGGSGGSEVQLVESGGGLVQPGGSLRLSCAASGFTFSTYAMNWVRQAPGKGLEWVGRIRSKYNNYATYYADSVKDRFTISRDDSKNSLYLQMNSLKTEDTAVYYCARHGNFGNSYVSWFAYWGQGTLVTVSS

SEQ ID NO: 134 - protein, 483 aa, synthetic construct
  REGION 1..483: note = Synthetic polypeptide
DIQMTQSPSSLSASVGDRVTITCRSSTGAVTTSNYANWVQQKPGKAPKALIGGTNKRAPGVPSRFSGSLIGDKATLTISSLQPEDFATYYCALWYSNLWVFGQGTKVEIKGGSGGSQVQLVQSGAEVKKPGASVKVSCKASGYTFTSYDINWVRQAPGQGLEWMGWMNPNSGNTGFAQKFQGRVTMTRDTSTSTVYMELSSLRSEDTAVYYCARDRAVTDYYYGMDVWGQGTLVTVSSGGSGQSVLTQPPSASGTPGQRVTISCSGSRSNIGSNTVNWYQQLPGTAPKLLIYGNNQRPSGVPDRFSGSKSGTSASLAISGLQSEDEADYYCATWDDSLIGWVFGGGTKLTVLGGSGGSEVQLVESGGGLVQPGGSLRLSCAASGFTFSTYAMNWVRQAPGKGLEWVGRIRSKYNNYATYYADSVKDRFTISRDDSKNSLYLQMNSLKTEDTAVYYCARHGNFGNSYVSYFAYWGQGTLVTVSS

SEQ ID NO: 135 - protein, 483 aa, synthetic construct
  REGION 1..483: note = Synthetic polypeptide
DIQMTQSPSSLSASVGDRVTITCRSSTGAVTTSNYANWVQQKPGKAPKGLIGGTNKRAPGVPSRFSGSLIGTDFTLTISSLQPEDFATYYCALWYSNLWVFGQGTKVEIKGGSGGSQVQLVQSGAEVKKPGASVKVSCKASGYTFTSYDINWVRQAPGQGLEWMGWMNPNSGNTGFAQKFQGRVTMTRDTSTSTVYMELSSLRSEDTAVYYCARDRAVTDYYYGMDVWGQGTLVTVSSGGSGQSVLTQPPSASGTPGQRVTISCSGSRSNIGSNTVNWYQQLPGTAPKLLIYGNNQRPSGVPDRFSGSKSGTSASLAISGLQSEDEADYYCATWDDSLIGWVFGGGTKLTVLGGSGGSEVQLVESGGGLVQPGGSLRLSCAASGFTFSTYAMNWVRQAPGKGLEWVGRIRSKYNNYATYYADSVKDRFTISRDDSKNSLYLQMNSLKTEDTAVYYCARHGNFGNSYVSWFAYWGQGTLVTVSS

SEQ ID NO: 136 - protein, 483 aa, synthetic construct
  REGION 1..483: note = Synthetic polypeptide
DIQMTQSPSSLSASVGDRVTITCRSSTGAVTTSNYANWVQQKPGKAPKALIGGTNKRAPGVPSRFSGSLIGDKATLTISSLQPEDFATYYCALWYSNLWVFGQGTKVEIKGGSGGSQVQLVQSGAEVKKPGASVKVSCKASGYTFTSYDINWVRQAPGQGLEWMGWMNPNSGNTGFAQKFQGRVTMTRDTSTSTVYMELSSLRSEDTAVYYCARDRANTDFSYGMDVWGQGTLVTVSSGGSGQSVLTQPPSASGTPGQRVTISCSGSRSNIGSNTVNWYQQLPGTAPKLLIYGNNQRPSGVPDRFSGSKSGTSASLAISGLQSEDEADYYCATWDDSLIGWVFGGGTKLTVLGGSGGSEVQLVESGGGLVQPGGSLRLSCAASGFTFSTYAMNWVRQAPGKGLEWVGRIRSKYNNYATYYADSVKDRFTISRDDSKNSLYLQMNSLKTEDTAVYYCARHGNFGNSYVSYFAYWGQGTLVTVSS

SEQ ID NO: 137 - protein, 483 aa, synthetic construct
  REGION 1..483: note = Synthetic polypeptide
DIQMTQSPSSLSASVGDRVTITCRSSTGAVTTSNYANWVQQKPGKAPKALIGGTNKRAPGVPSRFSGSLIGDKATLTISSLQPEDFATYYCALWYSNLWVFGQGTKVEIKGGSGGSQVQLVQSGAEVKKPGASVKVSCKASGYTFTSYDINWVRQAPGQGLEWMGWMNPNSGNTGFAQKFQGRVTMTRDTSTSTVYMELSSLRSEDTAVYYCARDRANTDYSFGMDVWGQGTLVTVSSGGSGQSVLTQPPSASGTPGQRVTISCSGSRSNIGSNTVNWYQQLPGTAPKLLIYGNNQRPSGVPDRFSGSKSGTSASLAISGLQSEDEADYYCATWDDSLIGWVFGGGTKLTVLGGSGGSEVQLVESGGGLVQPGGSLRLSCAASGFTFSTYAMNWVRQAPGKGLEWVGRIRSKYNNYATYYADSVKDRFTISRDDSKNSLYLQMNSLKTEDTAVYYCARHGNFGNSYVSYFAYWGQGTLVTVSS

SEQ ID NO: 138 - protein, 483 aa, synthetic construct
  REGION 1..483: note = Synthetic polypeptide
DIQMTQSPSSLSASVGDRVTITCRSSTGAVTTSNYANWVQQKPGKAPKALIGGTNKRAPGVPSRFSGSLIGDKATLTISSLQPEDFATYYCALWYSNLWVFGQGTKVEIKGGSGGSQVQLVQSGAEVKKPGASVKVSCKASGYTFTSYDINWVRQAPGQGLEWMGWMNPNSGNTGFAQKFQGRVTMTRDTSTSTVYMELSSLRSEDTAVYYCARDRANTDYSLGMDVWGQGTLVTVSSGGSGQSVLTQPPSASGTPGQRVTISCSGSRSNIGSNTVNWYQQLPGTAPKLLIYGNNQRPSGVPDRFSGSKSGTSASLAISGLQSEDEADYYCATWDDSLIGWVFGGGTKLTVLGGSGGSEVQLVESGGGLVQPGGSLRLSCAASGFTFSTYAMNWVRQAPGKGLEWVGRIRSKYNNYATYYADSVKDRFTISRDDSKNSLYLQMNSLKTEDTAVYYCARHGNFGNSYVSYFAYWGQGTLVTVSS

SEQ ID NO: 139 - protein, 481 aa, synthetic construct
  REGION 1..481: note = Synthetic polypeptide
DIQMTQSPSSLSASVGDRVTITCRSSTGAVTTSNYANWVQQKPGKAPKALIGGTNKRAPGVPSRFSGSLIGDKATLTISSLQPEDFATYYCALWYSNLWVFGQGTKVEIKGGSGGSQVQLVQSGAEVKKPGESLKISCKGSGYSFTSYWIGWVRQMPGKGLEWMGIIYPGDSDTRYSPSFQGQVTISADKSISTAYLQWSSLKASDTAMYYCARHKRGSDAFDIWGQGTTVTVSSGGSGQSVLTQPPSVSGAPGQRVTISCTGSSSNIGAGYDVHWYQQLPGTAPKLLIYGNSNRPSGVPDRFSGSKSGTSASLAITGLQAEDEADYYCQSYDSSLSDVVFGGGTKLTVLGGSGGSEVQLVESGGGLVQPGGSLRLSCAASGFTFSTYAMNWVRQAPGKGLEWVGRIRSKYNNYATYYADSVKDRFTISRDDSKNSLYLQMNSLKTEDTAVYYCARHGNFGNSYVSYFAYWGQGTLVTVSS

SEQ ID NO: 140 - protein, 481 aa, synthetic construct
  REGION 1..481: note = Synthetic polypeptide
EVQLVESGGGLVQPGGSLRLSCAASGFTFSTYAMNWVRQAPGKGLEWVGRIRSKYNNYATYYADSVKDRFTISRDDSKNSLYLQMNSLKTEDTAVYYCARHGNFGNSYVSYFAYWGQGTLVTVSSGGSGGSQSVLTQPPSVSGAPGQRVTISCTGSSSNIGAGYDVHWYQQLPGTAPKLLIYGNSNRPSGVPDRFSGSKSGTSASLAITGLQAEDEADYYCQSYDSSLSDVVFGGGTKLTVLGGSGQVQLVQSGAEVKKPGESLKISCKGSGYSFTSYWIGWVRQMPGKGLEWMGIIYPGDSDTRYSPSFQGQVTISADKSISTAYLQWSSLKASDTAMYYCARHKRGSDAFDIWGQGTTVTVSSGGSGGSDIQMTQSPSSLSASVGDRVTITCRSSTGAVTTSNYANWVQQKPGKAPKALIGGTNKRAPGVPSRFSGSLIGDKATLTISSLQPEDFATYYCALWYSNLWVFGQGTKVEIK

SEQ ID NO: 141 - protein, 484 aa, synthetic construct
  REGION 1..484: note = Synthetic polypeptide
DIQMTQSPSSLSASVGDRVTITCRSSTGAVTTSNYANWVQQKPGKAPKALIGGTNKRAPGVPSRFSGSLIGDKATLTISSLQPEDFATYYCALWYSNLWVFGQGTKVEIKGGSGGSQVQLVQSGAEVKKPGASVKVSCKASGYTFTSYYMHWVRQAPGQGLEWMGIINPSGGSTSYAQKFQGRVTMTRDTSTSTVYMELSSLRSEDTAVYYCARDVVPAAIDYYGMDVWGQGTTVTVSSGGSGQSVLTQPPSASGTPGQRVTISCSGSSSNIGSNTVNWYQQLPGTAPKLLIYSDNQRPSGVPDRFSGSKSGSSASLAISGLQSDDEADYYCATWDDSLNGAVFGGGTKLTVLGGSGGSEVQLVESGGGLVQPGGSLRLSCAASGFTFSTYAMNWVRQAPGKGLEWVGRIRSKYNNYATYYADSVKDRFTISRDDSKNSLYLQMNSLKTEDTAVYYCARHGNFGNSYVSYFAYWGQGTLVTVSS

SEQ ID NO: 142 - protein, 484 aa, synthetic construct
  REGION 1..484: note = Synthetic polypeptide
DIQMTQSPSSLSASVGDRVTITCRSSTGAVTTSNYANWVQQKPGKAPKGLIGGTNKRAPGVPSRFSGSLIGTDFTLTISSLQPEDFATYYCALWYSNLWVFGQGTKVEIKGGSGGSQVQLVQSGAEVKKPGASVKVSCKASGYTFTSYYMHWVRQAPGQGLEWMGIINPSGGSTSYAQKFQGRVTMTRDTSTSTVYMELSSLRSEDTAVYYCARDVVPAAIDYYGMDVWGQGTTVTVSSGGSGQSVLTQPPSASGTPGQRVTISCSGSSSNIGSNTVNWYQQLPGTAPKLLIYSDNQRPSGVPDRFSGSKSGSSASLAISGLQSDDEADYYCATWDDSLNGAVFGGGTKLTVLGGSGGSEVQLVESGGGLVQPGGSLRLSCAASGFTFSTYAMNWVRQAPGKGLEWVGRIRSKYNNYATYYADSVKDRFTISRDDSKNSLYLQMNSLKTEDTAVYYCARHGNFGNSYVSWFAYWGQGTLVTVSS

SEQ ID NO: 143 - protein, 483 aa, synthetic construct
  REGION 1..483: note = Synthetic polypeptide
DIQMTQSPSSLSASVGDRVTITCRSSTGAVTTSNYANWVQQKPGKAPKALIGGTNKRAPGVPSRFSGSLIGDKATLTISSLQPEDFATYYCALWYSNLWVFGQGTKVEIKGGSGGSQVQLVQSGAEVKKPGSSVKVSCKASGGTFSSYAISWVRQAPGQGLEWMGGIYPIFGSANYAQKFQGRVTITADESTSTAYMELSSLRSEDTAVYYCAREYYYDSSEWAFDIWGQGTLVTVSSGGSGQSVLTQPPSASGTPGQRVTISCSGSSSNIGSNIVNWYQQLPGTAPKLLIYSNNQRPSGVPDRFSGSKSGTSASLAISGLQSEDEADYYCAAWDDSLKGYVFGGGTKLTVLGGSGGSEVQLVESGGGLVQPGGSLRLSCAASGFTFSTYAMNWVRQAPGKGLEWVGRIRSKYNNYATYYADSVKDRFTISRDDSKNSLYLQMNSLKTEDTAVYYCARHGNFGNSYVSYFAYWGQGTLVTVSS

SEQ ID NO: 144 - protein, 483 aa, synthetic construct
  REGION 1..483: note = Synthetic polypeptide
DIQMTQSPSSLSASVGDRVTITCRSSTGAVTTSNYANWVQQKPGKAPKALIGGTNKRAPGVPSRFSGSLIGDKATLTISSLQPEDFATYYCALWYSNLWVFGQGTKVEIKGGSGGSQVQLVQSGAEVKKPGSSVKVSCKASGGTFSSYGISWVRQAPGQGLEWMGGIIPIFGSAHYAQKFQGRVTITADESTSTAYMELSSLRSEDTAVYYCAREYYYDSSEWAFDIWGQGTLVTVSSGGSGQSVLTQPPSASGTPGQRVTISCSGSSSNIGSNTVKWYQQLPGTAPKLLIYSNNQRSSGVPDRFSGSKSGTSASLAISGLQSEDEADYYCAAWDDSLNGYVFGGGTKLTVLGGSGGSEVQLVESGGGLVQPGGSLRLSCAASGFTFSTYAMNWVRQAPGKGLEWVGRIRSKYNNYATYYADSVKDRFTISRDDSKNSLYLQMNSLKTEDTAVYYCARHGNFGNSYVSYFAYWGQGTLVTVSS

SEQ ID NO: 145 - protein, 483 aa, synthetic construct
  REGION 1..483: note = Synthetic polypeptide
DIQMTQSPSSLSASVGDRVTITCRSSTGAVTTSNYANWVQQKPGKAPKGLIGGTNKRAPGVPSRFSGSLIGTDFTLTISSLQPEDFATYYCALWYSNLWVFGQGTKVEIKGGSGGSQVQLVQSGAEVKKPGSSVKVSCKASGGTFSSYGISWVRQAPGQGLEWMGGIIPIFGSAHYAQKFQGRVTITADESTSTAYMELSSLRSEDTAVYYCAREYYYDSSEWAFDIWGQGTLVTVSSGGSGQSVLTQPPSASGTPGQRVTISCSGSSSNIGSNTVKWYQQLPGTAPKLLIYSNNQRSSGVPDRFSGSKSGTSASLAISGLQSEDEADYYCAAWDDSLNGYVFGGGTKLTVLGGSGGSEVQLVESGGGLVQPGGSLRLSCAASGFTFSTYAMNWVRQAPGKGLEWVGRIRSKYNNYATYYADSVKDRFTISRDDSKNSLYLQMNSLKTEDTAVYYCARHGNFGNSYVSWFAYWGQGTLVTVSS

SEQ ID NO: 146 - protein, 483 aa, synthetic construct
  REGION 1..483: note = Synthetic polypeptide
DIQMTQSPSSLSASVGDRVTITCRSSTGAVTTSNYANWVQQKPGKAPKALIGGTNKRAPGVPSRFSGSLIGDKATLTISSLQPEDFATYYCALWYSNLWVFGQGTKVEIKGGSGGSQVQLVQSGAEVKKPGSSVKVSCKASGGTFDSYAISWVRQAPGQGLEWMGGIIPIFGSAHYSQKFQGRVTITADESTSTAYMELSSLRSEDTAVYYCAREYYYDSSEWAFDIWGQGTLVTVSSGGSGQSVLTQPPSASGTPGQRVTISCSGSSSNIGDNVVNWYQQLPGTAPKLLIYSTNKRPSGVPDRFSGSKSGSSASLAISGLQSEDEADYYCAAWDDSLSAYVFGGGTKLTVLGGSGGSEVQLVESGGGLVQPGGSLRLSCAASGFTFSTYAMNWVRQAPGKGLEWVGRIRSKYNNYATYYADSVKDRFTISRDDSKNSLYLQMNSLKTEDTAVYYCARHGNFGNSYVSYFAYWGQGTLVTVSS